European Patent Specification EP 3 743 726 B1, published June 12, 2024. Title: ANTIBODY, FUNCTIONAL FRAGMENT OR PROBE THEREOF AGAINST TUMOUR ANTIGENS. Applicant: Universidade NOVA de Lisboa Instituto Português de Oncologia do Porto FG, EPE Helmholtz-Zentrum Desden-Rossendorf, Institute of Radiopharmaceutical Cancer Research. The sequence listing filed with the application follows.

SEQUENCE LISTING (16 sequences)

SEQ ID NO: 1 - DNA, 339 bp, Mus musculus
gaagtgcagctgcaggagtccggacctggcctcgtgaaaccttctcagtctctgtctctcacctgctctgtcattggctactccatcaccagtggttattactggaactggatccggcagtttccaggaaacaaactggaatggatgggctccataaactacgacggtagcaatatctacaatccatctctcaaagatcgaatctccatcactcgtgacacatctaagaaccagtttttcctgaagttgaattctgtgactactgaggacacagctacatattactgtgcaagagggggggactactggggtcaaggaacctcagtcaccgtctcctca

SEQ ID NO: 2 - DNA, 351 bp, Mus musculus
gatattgtgctgacccagactccagcaatcatgtctgcatctccaggggagaaggtcaccttgacctgcagtgccagctcaagtgtaagttacatgcactggttccagcaaaagtcaggcacctcccccaaaagatggatttatgacacatccaaactggcttctggagtccctgctcgcttcagtggcagtgggtctgggacctcttactctctcacaatcagcagcatggaggctgaggatgctgccgcttattactgccagcagtggagtagtgacccacccatgctcacgttcggtgctgggaccaagctggagctgaaacgggctgatgctgcaccaactgtatcc

SEQ ID NO: 3 - protein, 113 aa, Mus musculus
EVQLQESGPGLVKPSQSLSLTCSVIGYSITSGYYWNWIRQFPGNKLEWMGSINYDGSNIYNPSLKDRISITRDTSKNQFFLKLNSVTTEDTATYYCARGGDYWGQGTSVTVSS

SEQ ID NO: 4 - protein, 107 aa, Mus musculus
IVLTQTPAIMSASPGEKVTLTCSASSSVSYMHWFQQKSGTSPKRWIYDTSKLASGVPARFSGSGSGTSYSLTISSMEAEDAAAYYCQQWSSDPPMLTFGAGTKLELK

SEQ ID NO: 5 - protein, 25 aa, Mus musculus
IVLTQTPAIMSASPGEKVTLTCSAS

SEQ ID NO: 6 - protein, 5 aa, Mus musculus
SSVSY

SEQ ID NO: 7 - protein, 17 aa, Mus musculus
MHWFQQKSGTSPKRWIY

SEQ ID NO: 8 - protein, 3 aa, Mus musculus
DTS

SEQ ID NO: 9 - protein, 36 aa, Mus musculus
KLASGVPARFSGSGSGTSYSLTISSMEAEDAAAYYC

SEQ ID NO: 10 - protein, 11 aa, Mus musculus
QQWSSDPPMLT

SEQ ID NO: 11 - protein, 25 aa, Mus musculus
EVQLQESGPGLVKPSQSLSLTCSVI

SEQ ID NO: 12 - protein, 9 aa, Mus musculus
GYSITSGYY

SEQ ID NO: 13 - protein, 17 aa, Mus musculus
WNWIRQFPGNKLEWMGS

SEQ ID NO: 14 - protein, 7 aa, Mus musculus
INYDGSN

SEQ ID NO: 15 - protein, 38 aa, Mus musculus
IYNPSLKDRISITRDTSKNQFFLKLNSVTTEDTATYYC

SEQ ID NO: 16 - protein, 6 aa, Mus musculus
ARGGDY